European Patent Application EP 4 442 264 A1, published October 9, 2024. Title: Therapeutic agent for diarrhea and method of treating diarrhea of cattle. Applicant: TOHOKU UNIVERSITY. The sequence listing filed with the application follows.

SEQUENCE LISTING (66 sequences)

SEQ ID NO: 1 - DNA, 425 bp, c__Bacteroidia
  source 1..425: mol_type = genomic DNA
atcctgtttgatccccacgctttcgtgcatcagcgtcaattgcggattcgtgagatgccttcgcaatcggtgttctgtgtgatatctatgcatttcaccgctacaccacacattcctcccacggcatccgcattctagcctaccagtatcaacggcacggtagaggttgagcccctaaatttcaccgctgacttaatagaccgcctacgcaccctttaaacccaataaatccggataacgcttgcatcccccgtattaccgcggctgctggcacggagttagccgatgcttattcgtaaggtactctcatcagcctacacgtagaccttattgctcccttacaaaagaagtttaagacccatagggccgtcaccttcacgcggcatggctggttcagtcgtcagaccattgaccaatattcctca

SEQ ID NO: 2 - DNA, 427 bp, f__Prevotellaceae
  source 1..427: mol_type = genomic DNA
aatcctgttcgatacccgcgctttcgagcttcagcgtcagttgcgccccagtgagctgccttcgcaatcggagttcttcgtgatatctaagcatttcaccgctacaccacgaattccgcccactttatgcgtactcaaggaaaccagttcgcgctgcagtgcagacgttgagcgtctacatttcacaacacgcttaatctccggcctacgctccctttaaacccaataaatccggataacgcccggaccttccgtattaccgcggctgctggcacggaattagccggtccttattcatagggtacatgcaaaaaaccacacgtggctcactttattcccctataaaagcagtttacaacccatagggccgtcttcctgcacgctacttggctggttcaggctctcgcccattgaccaatattcctca

SEQ ID NO: 3 - DNA, 426 bp, g__Prevotella
  source 1..426: mol_type = genomic DNA
atcctgttcgatacccgcactttcgagcttcagcgtcagttgcgctccagtgagctgccttcgcaatcggagttcttcgtgatatctaagcatttcaccgctacaccacgaattccgcccactttgtgcgtactcaaggaaaccagttcgcgctgcagtgcagacgttgagcgtctacatttcacaacacgcttaatctccggcctacgctccctttaaacccaataaatccggataacgcccggaccttccgtattaccgcggctgctggcacggaattagccggtccttattcataaggtacatgcaaaaagtctcacgagactcactttattcccttataaaagcagtttacaacccatagggccgtcttcctgcacgctacttggctggttcaggctctcgcccattgaccaatattcctca

SEQ ID NO: 4 - DNA, 431 bp, g__Succinispira
  source 1..431: mol_type = genomic DNA
aatcccgttcgctaccctggctttcgcatctcagcgtcagacacagtccagaaaggcgccttcgccaccggtgttcttcccaatatctacgcatttcaccgctacactgggagttcccctttcctctcctgcactcaagtcccccagtttcgatcgccatacggcgttaagcaccgcattttcacgaccgacttaaggaaccgcctacatgcgctttacgcccaataattccggacaacgcttgccacctacgtattaccgcggctgctggcacgtagttagccgtggcttcctcgttcactaccgtcactggaaacccatttcctggtccccccgttcgtcgtgaacaacagagttttacgttccgaagaacttcatcactcacgcggcgttgctccgtcaggctttcgcccattgcggaagattcccca

SEQ ID NO: 5 - DNA, 432 bp, g__Selenomonas
  source 1..432: mol_type = genomic DNA
atcctgttcgctccccacgctttcgagcctcagcgtcagttacagtccagaaagccgccttcgccactggtgttcctcctaatatctacgcatttcaccgctacactaggaattccgctttcctctcctgcactcaagaaagatagtttccatcccctcacggggttgagccccgcacttttaagatagacttaccttcccgcctgcgctccctttacgcccaataattccggacaacgctcgccacctacgtattaccgcggctgctggcacgtagttagccgtggcttcctcgtcaggtaccgtcattcagaacccatattctgagtcctgacattcgtccccgacaacagagctttacgagtcgaaacccttcttcactcacgcggcgttgctccgtcaggcttgcgcccattgcggaagattccccac

SEQ ID NO: 6 - DNA, 407 bp, g__Gemmiger
  source 1..407: mol_type = genomic DNA
atcctgtttgctacccatgctttcgagcctcagcgtcagttggtgcccagtaggtcgccttcgccactggtgttcctcccgatatctacgcattccaccgctacaccgggaattccacctacctctgcactactcaaggccagcagttttgaaagcaatttatgggttgagcccatagttttcacttccaacttgccggtccgcctgcgctccctttacacccagtaattccggacaacgcttgcaccctacgttttaccgcggctgctggcacgtagttagccggtgctttcttgttaggtaccgtcattatcgtccctaacgacaggagtttacaatccgaaaaccttcttcctccacgcggcgtcgctgcatcagggtttcccccattgtgcaatatcccccac

SEQ ID NO: 7 - DNA, 426 bp, g__Odoribacter
  source 1..426: mol_type = genomic DNA
atcctgttcgctacccacgctctcgtgcttcagcgtcagtcacagtctggtaagctgccttcgctatcggagttctaagttatatctaagcatttcaccgctacttaacttattccgcctacctcgtctgtactcaagctgaccagtattaatggctggccaaggtttagccatgacattttaccactaacttaatcaaccgcctacgcaccctttaaacccaataaatccggataacgctcgcatcctccgtattaccgcggctgctggcacggagttagccgatgcttattcattcggtacaggcatcgttccacgcgtgaaacttattcttcccgaataaaagaggtttacaacccatagggcagtcttccctcacgcgacttggctggttcagccttccggccattgaccaatattcctcac

SEQ ID NO: 8 - DNA, 431 bp, g__Lactobacillus
  source 1..431: mol_type = genomic DNA
atcctgtttgctacccacgctttcgaacctcagcgtcagttacagaccagagagccgctttcgccactggtgttcttccatatatctacgcatttcaccgctacacatggagttccactctcctcttctgcactcaagtcttccagtttccaatgcactactccggttaagccgaaggctttcacatcagacttaaaagaccgcctgcgttccctttacgcccaataaatccggacaacgcttgccacctacgtattaccgcggctgctggcacgtagttagccgtgacttgctggttagataccgtcatcgaatgaacagttactctcactcgtgttcttctctaacaacagagttttacgatccgaagaccttcttcactcacgcggcgttgctccatcagacttgcgtccattgtggaagattcccta

SEQ ID NO: 9 - DNA, 435 bp, o__Lactobacillales
  source 1..435: mol_type = genomic DNA
atcctgttcgctccccacgctttcgagcctcagcgtcagttacagaccagagagccgccttcgccactggtgttcctccatatatctacgcatttcaccgctacacatggaattccactctcctcttctgcactcaagtctcccagtttccaatgaccctccccggttgagccgggggctttcacatcagacttaagaaaccgcctgcgctcgctttacgcccaataaatccggacaacgcttgccacctacgtattaccgcggctgctggcacgtagttagccgtggctttctggttagataccgtcaagggatgaacattctcttctcatccttgttcttctctaacaacagagttttacgatccgaaaaccttcttcactcacgcggcgttgctcggtcagactttcgtccattgccgaagattccctactg

SEQ ID NO: 10 - DNA, 432 bp, f__Veillonellaceae
  source 1..432: mol_type = genomic DNA
aatcccgttcgctaccctggctttcgcatctcagcgtcagacacagtccagaaaggcgccttcgccaccggtgttcttcccaatatctacgcatttcaccgctacactgggagttcccctttcctctcctgcactcaagtgccacagtttccatcgccatacggggttaggccccgcagtttcacgacagacttaaggcaccgcctacatgcgctttacgcccaataattccggacaacgcttgccacctacgtattaccgcggctgctggcacgtagttagccgtggcttcctcgtacactaccgtcattgcttcccgttgttgatagaaagcacgttcgtcatgtacaacagggctttacgttccgaagaacttcctcacccacgcggcgttgctccgtcaggctttcgcccattgcggaagattcccca

SEQ ID NO: 11 - DNA, 432 bp, g__Acidaminococcus
  source 1..432: mol_type = genomic DNA
aatcccgtttgctaccctggctttcgcatctcagcgtcagacacagtccagaaaggcgccttcgccactggtgttcctcccaatatctacgcatttcaccgctacactgggaattcccctttcctctcctgcactcaagacttccagtatccaacgccatacggggttaagccccgcattttcacgtcggacttaaaagcccgcctacatgctctttacgcccaataattccggacaacgcttgccacctacgtattaccgcggctgctggcacgtagttagccgtggcttcctcgtcaggtaccgtcaacaccaaaatgtattatagatcggtgctttcgtccctgacaacagagttttacaacccgaaggccttcatcactcacgcggcgttgctccgtcagactttcgtccattgcggaagattcccca

SEQ ID NO: 12 - DNA, 408 bp, g__Collinsella
  source 1..408: mol_type = genomic DNA
aatcctgttcgctcccccagctttcgcgcctcagcgtcggtctcggcccagagggccgccttcgccaccggtgttccacccgatatctgcgcattccaccgctacaccgggtgttccaccctcccctaccggacccaagccgcggaggttccgggggcttcggggggttgagccccccgcttcgacccccggcctgccgggccgcctacgcgcgctttacgcccaatgaatccggataacgctcgccccctacgtattaccgcggctgctggcacgtagttagccggggcttcttctgcaggtacagtcttgactcttccctgctgaaagcggtttacgacccgaaggcctccatcccgcacgcggcgtcgctgcgtcagggttgcccccattgcgcaagattcccca

SEQ ID NO: 13 - DNA, 409 bp, g__Sporobacter
  source 1..409: mol_type = genomic DNA
aatcctgtttgctccccacgctttcgcgcctcaccgtcagttgtcgtccagtcatccgccttcgccactggtgttcttccttatatctacgcatttcaccgctacacaaggaattccgatgacctctccgatactcaagagaaacagtttcaaatgcagtttggaggttgagcctccagatttcacatctgacttgtctccccggctacacgccctttacacccagtaaatccggacaacgcttgccacctacgtattaccgcggctgctggcacgtagttagccgtggcttgttttcagggtaccgtcttctgctcttcccctgtcaaagaagtttacaacccgaaagccttcttccttcacgcggcgttgctgggtcagacttgcgtccattgcccaatattcccca

SEQ ID NO: 14 - DNA, 408 bp, c__Clostridia
  source 1..408: mol_type = genomic DNA
aatcctgtttgctccccacactttcgtgcctcaacgtcagtttctgtccagaaagtcgccttcgccactggtgttcctcctaatatctacgcatttcaccgctacactaggaattccactttcctctccagtactcaagaaaaacagtttcggttgcagttcctcagttaagccgagggatttcacaaccaacttattttcccgtctacgcaccctttacacccaataaatccggataacgctcgctccctacgtattaccgcggctgctggcacgtagttagccggagcttattctacaggtactgtcttgtttcttccctgtctaaagcagtttacaatccgaaaaccttcttcctgcacgcggcgtcactgcgtcagagtttcctccattgcgcaatattcccga

SEQ ID NO: 15 - DNA, 433 bp, g__Treponema
  source 1..433: mol_type = genomic DNA
aatcctgtttgctccccgcaccttcgcacctcagcgtcagtaatctgctggtagcctgccttcgccattggtgttcttccagatatctacagatttcacccctacacctggaattccggctgcccctcagttactctagtcgtgcagttctcaacgcagtgccggagttaagccccggcatttcacaccaagcttgcacaaccgcctacatgccctttacgcccaataattccgaacaacgctcggggcttacgtgttaccgcggctgctggcacgtaattagccgccccttattcaagtgctacggtcatcttcttaccatttcctgtaaactttattcatcacactcaaaaggattttacaaccttccggccttcatcatccacgcggcgtcgctccgtcagagtttcctccattgcggaatattcttagc

SEQ ID NO: 16 - DNA, 430 bp, p__Tenericutes
  source 1..430: mol_type = genomic DNA
atcctgtttgctccccacgctttcgtgcctcagcgtcagtaatggcccagcaagccgccttcgccactggtgttcttccatatatttacgaattttacctctacacatggagttccacttgcctctaccacactctagtttgccagtatccaaggcatcacggggttgagccccgcacttttacctcagacttaacataccgcctacgcaccctttacgcccaataattccggataacgcttgctccctacgtattaccgcggctgctggcacgtagttagccggagcttattcgtaaagtaccgtcattcactacccatttcctgatagtgctgttcgtcctctacaaaagaattttacataccgaaatacttcatcattcacgcggcgttgctcggtcagggtttcccccattgccgaaaattcccta

SEQ ID NO: 17 - DNA, 434 bp, o__Spirochaetales
  source 1..434: mol_type = genomic DNA
taatcctgtttgctccccgcaccttcgcacctcagcgtcagtcatctgcccgaaacttgccttcgccattggtgttcttccagatatctgcagatttcacccctacacctggaattccagtttcgcctcagagactcaagccctgtagttctcaatgcagtccacaggttgagcctgtggatttcacaccaagcttgcagggccgcctacatgccctttatgcccaataattccgaacaacgctcgcaacttacgtgttaccgcggctgctggcacgtaattagccgttgcttattcaggacctaccgtcaccacaatgccattccctgcactgcttattcttcagtcccaaaaggattttacaaccttccggccttcctcatccacgcggcgtcgctccgtcagactttcgtccattgcggaatattcttagc

SEQ ID NO: 18 - DNA, 427 bp, g__CF231
  source 1..427: mol_type = genomic DNA
aatcctgtttgatacccgcactttcgagcctcagcgtcaatagcaccccaggagactgccttcgcaatcggagttcttcgtcatatctaagcatttcaccgctacacgacgaattccatctcccttgtgtgcattcaagaccgccagtttcaacggcaggacaaggttgggccttgacattttaccgctgacttaacagtccgcctacgctccctttaaacccaataaatccggataacgctcgcatcttccgtattaccgcggctgctggcacggaattagccgatgcttattcgtaaggtacatgcaaaatactacacgtagtatcatttattcccaaacaaaagaagtttacaacccgtagggcagtcatccttcacgctacttggctggttcaggctctcgcccattgaccaatattcctcac

SEQ ID NO: 19 - DNA, 408 bp, k__Bacteria
  source 1..408: mol_type = genomic DNA
atcctgtttgctccccacgctttcgtgcctgagcgtcagttatggtccagaaagccgccttcgctactggtgttcctccgaatctctacgcatttcaccgctacactcggaattccactttcctctcccacactctagcctagcagtttcagaagcagctccggggttgagccccgaaatttcacttctgacttaccaggccgcctgcgcaccctttacacccagtaaatccggataacgctcgctccctacgtattaccgcggctgctggcacgtagttagccggagcttcttagtcaggtaccgtcatttattcttccctgctgatagaagtttacaatccgaagaccttcatccttcacgcggcgtcgctgcatcaggcttgcgcccattgtgcaatattcccca

SEQ ID NO: 20 - DNA, 432 bp, p__Spirochaetes
  source 1..432: mol_type = genomic DNA
aatcctgtttgctccccacaccttcgcacctcagcgtcagttatctgcctgaaacctgccttcgccattggtattcttccagatatctacagatttcacccctacacctggaattctgattccacttcagtaactctagctacccagttctcagtgcagtccaagagttgagctcttgcctttcacaccaagcttaggtaaccgcctacatgccctttacgcccaataattccgaacaacgctcgcaacttacgtgttaccgcggctgctggcacgtaattagccgttgcttattcaaattgtaccgtcaccactatatcattccctacatagcttattcgtccaattcaaaaggattttacaacctttcggccttcttcatccacgcggcgtcgctccgtcagactttcgtccattgcggaatattcttag

SEQ ID NO: 21 - DNA, 409 bp, g__Roseburia
  source 1..409: mol_type = genomic DNA
aatcctgtttgctccccacgctttcgagcctcagcgtcagttatcgtccagtaagccgccttcgccactggtgttcctcctaatatctacgcatttcaccgctacactaggaattccgcttacccctccgacactctagcacgacagtttccaatgcagtaccggggttgagccccgggctttcacatcagacttgccgcgccgcctgcgctccctttacacccagtaaatccggataacgcttgcaccatacgtattaccgcggctgctggcacgtatttagccggtgcttcttagtcaggtaccgtcattcttcttccctgctgatagaactttacataccgaaatacttcttcattcacgcggcgtcgctgcatcaggctttcgcccattgtgcaatattccccac

SEQ ID NO: 22 - DNA, 426 bp, g__Alistipes
  source 1..426: mol_type = genomic DNA
atcctgtttgctccccacgctttcgtgcctcagcgtccgaaaagagtttgtgagctgctttcgcaatcggtgttctgtgtaatctctaagcatttcaccgctacactacacattccgcccacagcactctctcgctagcccaacagtatcagaggcacgtccatcgttgagcgatgggatttcacctctaacttaccaggccgcctacgcaccctttaaacccaataaatccggataacgctcggatcctccgtattaccgcggctgctggcacggagttagccgatccttattcttgcgatactttcagacaggtacacgtacctgcgtttaccctcgcataaaagcagtttacaactcatagagccgtcttcctgcacgcggcatggctggttcagacttgcgtccattgaccaatattcctca

SEQ ID NO: 23 - DNA, 408 bp, g__Lactonifactor
  source 1..408: mol_type = genomic DNA
aatcctgtttgctccccacgctttcgagcctcaacgtcagtcatcgtccagtaagccgccttcgccactggtgttcctcctaatatctacgcatttcaccgctacactaggaattccacttacctctccgacactctagtctaacagtttccaatgcagttccggggttgagccccggattttcacatcagacttgccagaccgtctacgctccctttacacccagtaaatccggataacgcttgcaccatacgtattaccgcggctgctggcacgtatttagccggtgcttcttagtcaggtaccgtcattttcttccctgctgatagagctttacataccgaaatacttcatcgctcacgcggcgtcgctgcatcagggtttcccccattgtgcaatattccccac

SEQ ID NO: 24 - DNA, 429 bp, Paraprevotellaceae
  source 1..429: mol_type = genomic DNA
taatcctgtttgatacccgcactttcgagcctcagcgtcagttgcaccccagatggctgccttcgcaatcggagttcttcgtgatatctaagcatttcaccgctacaccacgaattccaccatccttatgtgcactcaagaaagccagtatcaactgcagttccgccgttgagcgacgggatttcacagctgacttaacattccgcctgcgctccctttaaacccaataaatccggataacgctcggaccttccgtattaccgcggctgctggcacggaattagccggtccttattcgtacggtacatgcaaaaaggctcacgagcctcactttattcccgtacaaaagaagtttacaacccgtagggcagtcttccttcacgctacttggctggttcaggctctcgcccattgaccaatattcctcac

SEQ ID NO: 25 - DNA, 430 bp, p__Tenericutes; identical to SEQ ID NO: 16
  source 1..430: mol_type = genomic DNA

SEQ ID NO: 26 - DNA, 408 bp, g__Lactonifactor; identical to SEQ ID NO: 23
  source 1..408: mol_type = genomic DNA

SEQ ID NO: 27 - DNA, 432 bp, p__Spirochaetes; identical to SEQ ID NO: 20
  source 1..432: mol_type = genomic DNA

SEQ ID NO: 28 - DNA, 433 bp, o__Spirochaetales; identical to SEQ ID NO: 15
  source 1..433: mol_type = genomic DNA

SEQ ID NO: 29 - DNA, 433 bp, g__Treponema; identical to SEQ ID NO: 15
  source 1..433: mol_type = genomic DNA

SEQ ID NO: 30 - DNA, 432 bp, c__Spirochaetes; identical to SEQ ID NO: 20
  source 1..432: mol_type = genomic DNA

SEQ ID NO: 31 - DNA, 426 bp, g__Alistipes; identical to SEQ ID NO: 22
  source 1..426: mol_type = genomic DNA

SEQ ID NO: 32 - DNA, 409 bp, g__Roseburia; identical to SEQ ID NO: 21
  source 1..409: mol_type = genomic DNA

SEQ ID NO: 33 - DNA, 410 bp, g__Succinivibrio
  source 1..410: mol_type = genomic DNA
atcctgtttgctacccacgctttcgcatatgagcgtcagtatttgcccaggagactgccttcgcctttggtgttcttccagatatctacgcattccaccgctacacctggaattccgtctccccctgcaatactctagtccaccagtttagtatgctgttcccaggttgagcccggggatttcacatcctacttgatgaaccgcctgcatgccctttacgcccagttattccgattaacgcttgcaccctccgtattaccgcggctgctggcacggagttagccggtgcttcttctgagggtaacgtcatttttttcctcccctccgaaagtgctttacaacccgaaggccttcttcacacacgcggcatggctgcatcagagtttcctccattgtgcaatattccctac

SEQ ID NO: 34 - DNA, 407 bp, g__Clostridium
  source 1..407: mol_type = genomic DNA
atcctgtttgctccccacgctttcgagcctcagcgtcagtaaaagcccagttggccgccttcgccactggtgttcctcctaatatctacgcatttcaccgctacactaggaattccgccaacctctacttcactcaagaaatgcagttttgaacgctgatatgggttgagcccatagattaaacattcaacttgcactcccgcctacgctccctttacacccagtaattccggacaacgctcgctccctacgtattaccgcggctgctggcacgtagttagccggagcttcctccttgggtaccgtcattatcgtccccaaagccagtggtttacaacccgagggccgtcttcccacacgcggcgtcgctgcatcaggcttgcgcccattgtgcaatatcccccact

SEQ ID NO: 35 - DNA, 428 bp, f__S24-7
  source 1..428: mol_type = genomic DNA
aatcctgttcgatacccacgccttcgtgcttcagcgtcagttgagcgccggtatgctgccttcgcaatcggagttctgcgtgatatctatgcatttcaccgctacaccacgcattccgcatacttctcgctcactcaagaacggcagtttcaacggctcgacggagttgagctccgcatttttaccgctgacttaccgtcccgcctacgcaccctttaaacccaataaatccggataacgctcgcatcctccgtattaccgcggctgctggcacggagttagccgatgctttttcttcgggtactctcgcttttagtcacacgtgacttctttgctccccgacaaaagaggtttacaatccataggaccgtcttccctcacgcgacttggctggttcaggctcccgcccattgaccaatattcctcac

SEQ ID NO: 36 - DNA, 425 bp, f__Barnesiellaceae
  source 1..425: mol_type = genomic DNA
aatcctgttcgatccccacgctttcgtgcctcagcgtcagatagatgccggcatgctgccttcgcaatcggagttctgcgtgatatctatgcatttcaccgctacaccacgcattccgcatacttctcatcctctctagctcatcagtttcaacggcaggccgaggttgagccccgacatttaaccgctgacttgacgtgccgcctacgcaccctttaaacccaataaatccggataacgctcgcatcctccgtattaccgcggctgctggcacggagttagccgatgctttttcttcaggtacactcatcttaccacgcgtggtctctttgttccctgacaaaagaggtttacaatacttagtaccgtcttccctcacgcgacttggctggttcaggctctcgcccattgaccaatattcctca

SEQ ID NO: 37 - DNA, 427 bp, o__Bacteroidales
  source 1..427: mol_type = genomic DNA
aatcctgttcgatacccacgctttcgtgcctcagcgtcagtagcgcgctcgacggctgccttcgcaatcggagttctgcgtgatatctatgcatttcaccgctacaccacgcattccgccatcgtcgcgcgcactccagcacatcagtatcaacggcggaacggggttgagccccgtcatttgaccgctgacttgacacgccgcctgcgcaccctttaaacccaataaatccggataacgctcgcatcctccgtattaccgcggctgctggcacggagttagccgatgcttattcgacgggtacgctcatcggcgtatgcatacgccttattgctccccgacaaaagaggtttacaatccgtaggaccttcctccctcacgcgacttggctggttcagacttccgtccattgaccaatattcctcac

SEQ ID NO: 38 - DNA, 430 bp, o__Aeromonadales
  source 1..430: mol_type = genomic DNA
atcctgtttgctacccacgctttcgcacctcagtgtcagtatctgtccaggaggccgccttcgcctctggtattcttccacatctctacgcatttcaccgctacacgtggaattctacctccctctacagtactccagttcaacagttttggatgcagtccccatgttaagcacgggaatttcacatccaacttatctcgccacctgcgtgccctttacgcccagtcattccgattaacgctcgcaccctccgtattaccgcggctgctggcacggagtttgccggtgcttattcacactctaacgtcaaatagcgcatttatttatacgctgtcttcctcgaatgcaaaagtgctttacaacccgaaggccttcttcacacacgcggcatggctgcatcagggtttcccccattgtgcaatattcccca

SEQ ID NO: 39 - DNA, 407 bp, f__Lachnospiraceae
  source 1..407: mol_type = genomic DNA
aatcctgtttgctccccacgctttcgagcctcaacgtcagtcatcgtccagtaagccgccttcgccactggtgttcctcccaatatctacgcatttcaccgctacactgggaattccacttacctctccgacactctagctgcatagtttccaaagcagtcccggggttgagccccgggctttcacttcagacttacacagccgtctacgctccctttacacccagtaaatccggataacgcttgcaccatacgtattaccgcggctgctggcacgtatttagccggtgcttcttagtcaggtaccgtcattttcttccctgctgatagagctttacataccgaaatacttcttcgctcacgcggcgtcgctgcatcagggtttcccccattgtgcaatattcccca

SEQ ID NO: 40 - DNA, 406 bp, f__Ruminococcaceae
  source 1..406: mol_type = genomic DNA
atcctgtttgctacccatgctttcgagcctcagcgtcagttagtgcccagtaggccgccttcgccactggtgttcctcccgatatctacgcattccaccgctacaccgggaattccgcctacctctacaccactcaagatcggcagttttgaaggcagtttgtgagttgagcccacagctttcacctccaacttgccgacccgcctgcgctccctttacacccagtaattccggacaacgcttgccacctacgttttaccgcggctgctggcacgtagttagccgtggcttcctcctcgggtaccgtcattatcgtccccgaagacaggagtttacaatccgaaaaccttcttcctccacgcggcgtcgctgcatcagggtttcccccattgtgcaatattcccca

SEQ ID NO: 41 - DNA, 408 bp, g__Eggerthella
  source 1..408: mol_type = genomic DNA
ctaatcctgttcgctcccccggctttcgcgcctcagcgtccttcagggcccagagagctgccttcgccgtcggtgttcttcccgatatctgcgcattccaccgctacaccgggaattccgctctcccctacccgaagcgagccgcccagttcgggacccggcccggggttgagccccgggattagaggtcccgcttgagcggccgcctgcgcgcgctttacgcccaatgaatccggataacgctcgccccctacgtgttaccgcggctgctggcacgtagttagccggggcttcttctgcaggtaccgtcgatgtcttccctgctgaaagcggtttacgacgcggacgccttcgtcccgcacgcggcgttgctgcgtcagggttgcccccattgcgcaatattcccca

SEQ ID NO: 42 - DNA, 432 bp, g__Anaerorhabdus
  source 1..432: mol_type = genomic DNA
taatcctatttgctccccacgctttcgtgcttcagcgtcagttacaggccagcagaccgccttcgccactggtgttcctccatatatctacgcattttaccgctacacatggaattccatctgcctctcctgcactccagtataccagtttccaaagcttgattgagttgagctcaacgattttacttcagacttaatataccgcctacgcaccctttacgcccaataattccggataacgcttgccacctacgtattaccgcggctgctggcacgtagttagccgtggctttctggtaaggtaccgtcacttacggatcattccctatccgtaccgttcttcccttacaacagagctttacaacccgaaggccgtcttcactcacgcggcattgctcggtcagggttccccccattgccgaaaattcccta

SEQ ID NO: 43 - DNA, 409 bp, g__Roseburia; identical to SEQ ID NO: 21
  source 1..409: mol_type = genomic DNA

SEQ ID NO: 44 - DNA, 391 bp, o__Methanobacteriales
  source 1..391: mol_type = genomic DNA
atccggttcgcgcccctggctttcgttactcaccgtcaagatcgttccagttagacgccttcgccacaggtggtcctcccaggattataggatttcacccctaccccggtagtacctctaacctctcccgacttcaagtctgatagtatctccagcaattcttatagttaagctacaagctttcaccaaagacttatcaaaccggctacgaacgctttaggcccaataaaaacagctaccactcgagctgccggtgttaccgcggcggctggcaccggtcttgcccagctcttattctaaaagctttttacactaatgaaaagttatacaaaaaagcataacacttgggatccccccgtcgcactttcgtacattgcggaggtttcgcgcc

SEQ ID NO: 45 - DNA, 391 bp, p__Euryarchaeota
  source 1..391: mol_type = genomic DNA
aatccggttcgcgcccctagctttcgtccctcaccgtcaggttcgttccagttagccgccttcgccacaggtggtcctcccaggattacagaatttcacctctaccctgggagtaccgctaacctctcccgacctcaagttcaacagtatcaccagcaattcccacagttaagctacaggatttcaccagtgacttatcaaaccggctacgaacgctttaggcccaataaaaacagctaccactagagctgccggtgttaccgcggcggctggcaccggtcttgcccagctcttattccaaaagctttttacacttaagaaaagccatcccgttaagaatggcacttgggatccccccgtcgcgatttctcacattgcggaggtttcgcgc

SEQ ID NO: 46 - DNA, 391 bp, c__Methanobacteria
  source 1..391: mol_type = genomic DNA
atccggttcgcgcccctaactttcgtccctcaccgtcagaaccgttccagttagacgccttcgcaacaggcggtcctcccaggattacagaatttcacctctaccctgggagtacctctaacctctcccggtctcaagtctaatagtatctccagcaattcccacagttaagctgcaggatttcaccagagacttattaaaccggctacggacgctttaggcccaataaaaattgttaccactagagctgccggtgttaccgcggcggctggcaccggtcttgcccagctcttattccaaaagctctttacactaatgaaaagccatcccgttaagaatggcacttgggatccccccgtcgcgatttctcacattgcggaggtttcgcgcc

SEQ ID NO: 47 - DNA, 391 bp, f__Methanobacteriaceae
  source 1..391: mol_type = genomic DNA
atccggttcgcgcccctaactttcgtccctcaccgtcagaaccgttccagttagacgccttcgcaacaggcggtcctcccaggattacagaatttcacctctaccctgggagtacctctaacctctcccggtctcaagtctaatagtatctccagctattcccacagttaagctacaggatttcaccagagacttattaaaccggctacggacgctttaggcccaataaaaactgctaccactagagctgccggtgttaccgcggcggctggcaccggtcttgcccagcccttattccaaaagctctttacactaatgaaaagccatcccgttaagaatggcacttgggatccccccgtcgcgatttctcacattgcggaggtttcgcgcc

SEQ ID NO: 48 - DNA, 391 bp, k__Archaea
  source 1..391: mol_type = genomic DNA
aatccggttcgcgcccctaactttcgtccctcaccgtcagaaccgttccagttagacgccttcgcaacaggcggtcctcccaggattacagaatttcacctctaccctgggagtacctctaacctctcccggtctcaagtctaatagtatctccagcaattcccacagttaagctacaggatttcaccagagacttattaaaccggctacggacgctttaggcccaataaaagttgctaccactagagctgccggtgttaccgcggcggctggcaccggtcttgcccagctcttattccaaaagctttttacactaatgaaaagccatcccgttaagaatggcacttgggatccccccgtcgcgatttctcacattgcggaggtttcgcgc

SEQ ID NO: 49 - DNA, 392 bp, g__Methanobrevibacter
  source 1..392: mol_type = genomic DNA
aatccggttcgcgcccctagctttcgtccctcaccgtcaggttcgttccagttagccgccttcgccacaggtggtcctcccaggattacagaatttcacctctaccctgggagtaccgctaacctctcccgacctcaagttcaacagtatcaccagcaattcccacagttaagctacaggatttcaccagagacttatcaaaccggctacgaacgctttaggcccaataaaaacagctaccactagagctgccggtgttaccgcggcggctggcaccggtcttgcccagctcttattccaaaagctttttacacttaagaaaagctatcccgttaagaatagcacttgggatccccccatcgcactctcgtacattgtggaggtttcgcgcc

SEQ ID NO: 50 - DNA, 407 bp, g__Clostridium; identical to SEQ ID NO: 34
  source 1..407: mol_type = genomic DNA

SEQ ID NO: 51 - DNA, 434 bp, f__bacillaceae
  source 1..434: mol_type = genomic DNA
aatcctgtttgctccccacgctttcgcgcctcagtgtcagttgcagaccagaaagtcgccttcgccaccggtgttcctccacatctctacgcatttcaccgctacacgtggaattccactttcctcttctgcactcaagtttcccagtttccaatgcagttctacggttgagccgtaggctttcacatcagacttaagaaaccacctgcgcgcgctttacgcccaataattccggataacgctcgccacctacgtattaccgcggctgctggcacgtagttagccgtggctttctcgttaggtaccgtcacgataccgccttattcaaacggtatttgttcttccctaacaacagaactttacgatccgaaaaccttcatcgttcacgcggcgttgctccgtcagactttcgtccattgcggaagattccctac

SEQ ID NO: 52 - DNA, 432 bp, f__Spirochaetaceae
  source 1..432: mol_type = genomic DNA
aatcctgtttgctccccacaccttcgcacctcagcgtcagtcatctgctggtaggctgccttcgccattggtattcttccagatatctacagatttcacccctacacctggaattctgcctgcccctcagtgactctagttatgcagttctcaacgcagtccaggagttaagctcctgcctttcacaccaagcttgcataaccgcctacatgccctttacgcccaataattccgaacaacgctcgcaacttacgtgttaccgcggctgctggcacgtaattagccgttgcttattcaagtactacagtcaccatagtgtcattccctacactacttattcctcatacttaaaaggattttacaaccttccggccttcttcatccacgcggcgtcgctccgtcagactttcgtccattgcggaatattcttag

SEQ ID NO: 53 - DNA, 432 bp, p__Spirochaetes; identical to SEQ ID NO: 20
  source 1..432: mol_type = genomic DNA

SEQ ID NO: 54 - DNA, 433 bp, g__Treponema; identical to SEQ ID NO: 15
  source 1..433: mol_type = genomic DNA

SEQ ID NO: 55 - DNA, 432 bp, c__Spirochaetes; identical to SEQ ID NO: 20
  source 1..432: mol_type = genomic DNA

SEQ ID NO: 56 - DNA, 433 bp, o__Spirochaetales; identical to SEQ ID NO: 15
  source 1..433: mol_type = genomic DNA

SEQ ID NO: 57 - DNA, 408 bp, f__F16
  source 1..408: mol_type = genomic DNA
atcccgtttgctccctacgctttcgtgccttagtgtcagaaacgccccagtaacctgcctacgctatcggtgttccttctaatatctacggatttcactcctacactagaaattccagttacccatgacgctctcgagacgtccagtttaggtaatagtctgaatggttgagccaccagatttcactacctacttaaacatccacctacgcaactctttacgcccagtcactccggataatgctcggatcctacgtatgaccgcggctgctggcacgtagttagccgatccttattcataagttaccatcatatttctcgcttataaaagcagtttacaacccgaaggccttcatcctgcacgcggcgttgctccatcaggctttcgcccattgtgaaagattcccta

SEQ ID NO: 58 - DNA, 408 bp, p__TM7
  source 1..408: mol_type = genomic DNA
atcccgtttgctccctacgctttcgtgccttagtgtcagaaatgtcccagtagcctgcctacgctatcggtgttctttctaatatctacggatttcactcctacactagaaattccagctacccctaacattctcgagcttggcagtttagataatagtctgaatggttgagccaccagatttcactatctacttaccatgccacctacgcaactctttacacccagtcaatccggataatgcttggaccctacgtatgaccgcggctgctggcacgtagttagccggtccttattcaaaacctaccatcatatttctcggttataaaagcagtttacaacccgaaggccgtcatcctgcacgcggcgttgctccatcaggctttcgcccattgtgaaagattcccta

SEQ ID NO: 59 - DNA, 432 bp, f__alcaligenaceae
  source 1..432: mol_type = genomic DNA
atcctgtttgctccccacgctttcgtgcatgagcgtcagtattatcccagggggctgccttcgccatcggtattcctccacatctctacgcatttcactgctacacgtggaattctacccccctctgacatactctagtccgggagttaaaaatgccattccaaggttgagccctgggatttcacatctttctttccgaaccgcctgcgcacgctttacgcccagtaattccgattaacgctcgcaccctacgtattaccgcggctgctggcacgtagttagccggtgcttattcttcaggtaccgtcagcgttttctggtattagcaaaaaacttttcttccctgacaaaagtgctttacaacccgaaggccttcatcgcacacgcgagatggctggatcagggtttcccccattgtccaaaattccccac

SEQ ID NO: 60 - DNA, 432 bp, o__Pasteurellales
  source 1..432: mol_type = genomic DNA
aatcctgtttgctccccacgctttcgcacatgagcgtcagtacatccccaaggggctgccttcgccttcggtattcctccacatctctacgcatttcaccgctacacgtggaattctacccctccctaaagtactctagacccccagtctgaaatgcaattcccaggttaagcccggggatttcacacctcacttaaaagtccgcctgcgtgccctttacgcccagttattccgattaacgctcgcaccctccgtattaccgcggctgctggcacggagttagccggtgcttcttctgtgactaacgtcaattgtatgctctattaaaacatccaccttcctcatcaccgaaagaactttacaacccgaaggccttcttcattcacgcggcatggctgcgtcagggttgcccccattgcgcaatattcccca

SEQ ID NO: 61 - DNA, 432 bp, f__Pasteurellaceae
  source 1..432: mol_type = genomic DNA
aatcctgtttgctccccacgctttcgcacatgagcgtcagtacattcccaaggggctgccttcgccttcggtattcctccacatctctacgcatttcaccgctacacgtggaattctacccctccctaaagtactctagactcccagtctgaaatgcaattcccaggttaagcccggggctttcacatcccacttaaaagtccgcctgcgtgccctttacgcccagttattccgattaacgctcgcaccccccgtattaccgcggctgctggcacggagttagccggtgcttcttctgtagttaacgtcaattgattgttctattaaaacaaccaccttcctcgctaccgaaagaactttacaacccgaaggccttcttcattcacgcggcatggctgcatcagggttccccccattgtgcaatattcccca

SEQ ID NO: 62 - DNA, 434 bp, p__Proteobacteria
  source 1..434: mol_type = genomic DNA
aatcctgtttgctccccacgctttcgcacctcagtgtcagtatcagtccaggtagtcgccttcgccactgatgttccttcctatatctacgcatttcaccgctacacaggaaattccactaccctctactgtactctagcctgctagttttgaaagcaattcccaggttgagcccggggctttcacttccaacttaacaaaccacctacgcgcgctttacgcccagtaattccgattaacgcttgcacccttcgtattaccgcggctgctggcacgaagttagccggtgcttattctgttggtaacgtcaaaacttagcgggtattaaccgtaagcccttcctcccaacttaaagtgctttacaatccgaagaccttcttcacacacgcggcatggctggatcagggtttcccccattgtccaatattccccac

SEQ ID NO: 63 - DNA, 432 bp, f__Enterobacteriaceae
  source 1..432: mol_type = genomic DNA
aatcctgtttgctccccacgctttcgcacctgagcgtcagtcttcgtccagggggccgccttcgccaccggtattcctccagatctctacgcatttcaccgctacacctggaattctacccccctctacgagactcaagcttgccagtatcagatgcagttcccaggttgagcccggggatttcacatctgacttaacaaaccgcctgcgtgcgctttacgcccagtaattccgattaacgcttgcaccctccgtattaccgcggctgctggcacggagttagccggtgcttcttctgcgggtaacgtcaatgagcaaaggtattaactttactcccttcctccccgctgaaagtactttacaacccgaaggccttcttcatacacgcggcatggctgcatcaggcttgcgcccattgtgcaatattcccca

SEQ ID NO: 64 - DNA, 432 bp, o__Enterobacteriales
  source 1..432: mol_type = genomic DNA
atcctgtttgctccccacgctttcgcacctgagcgtcagtctttgtccagggggccgccttcgccaccggtattcctccagatctctacgcatttcaccgctacacctggaattctacccccctctacaagactctagcctgccagtttcgaatgcagttcccaggttgagcccggggatttcacatccgacttgacagaccgcctgcgtgcgctttacgcccagtaattccgattaacgcttgcaccctccgtattaccgcggctgctggcacggagttagccggtgcttcttctgcgggtaacgtcaatcgccaaggttattaaccttaacgccttcctccccgctgaaagtgctttacaacccgaaggccttcttcacacacgcggcatggctgcatcaggcttgcgcccattgtgcaatattccccac

SEQ ID NO: 65 - DNA, 428 bp, f_Bacteroidaceae
  source 1..428: mol_type = genomic DNA
aatcctgtttgatacccgcactttcgagcctcaacgtcagtggcggcttagcaggctgccttcgcaatcggggttcttcgtgatatctaagcatttcaccgctacaccacgaattccgcctgcctcaaccgtactcaaggtctccagtttcaactgcaattttaaggttgagccccaaactttcacagctgacttaaaaacccgtctacgctccctttaaacccaataaatccggataacgctcgcatcctccgtattaccgcggctgctggcacggagttagccgatgcttattcgttacggtacatgcaaaaacctacacgtaggttcctttattcccgcacaaaagaagtttacaacccgtagggccgtcatccttcacgctacttggctggttcaggctctcgcccattgaccaatattcctca

SEQ ID NO: 66 - DNA, 427 bp, g_Bacteroides
  source 1..427: mol_type = genomic DNA
aatcctgtttgatacccacactttcgagcctcaatgtcagttgcagcttagcaggctgccttcgcaatcggagttcttcgtgatatctaagcatttcaccgctacaccacgaattccgcctgcctcaactgcactcaagatatccagtatcaactgcaattttacggttgagccgcaaactttcacaactgacttaaacatccatctacgctccctttaaacccaataaatccggataacgctcggatcctccgtattaccgcggctgctggcacggagttagccgatccttattcataaagtacatgcaaacgggtatgcatacccgactttattcctttataaaagaagtttacaacccatagggcagtcatccttcacgctacttggctggttcaggctctcgcccattgaccaatattcctca